European Patent Application EP 4 298 902 A1, published January 3, 2024. Title: 一种基于基因改造脊椎动物的携带通用定点偶联接口的抗体的制备方法. Applicant: 苏州有诺真生物科技有限公司. The sequence listing filed with the application follows.

SEQUENCE LISTING (5 sequences)

SEQ ID NO: 1 - DNA, 23 bp, Artificial sequence
  Synthesized
ggaatgagtgttagagacaaagg

SEQ ID NO: 2 - DNA, 306 bp, Artificial sequence
  Synthesized
atgagcagcaccctcacgttgaccaaggacgagtatgaacgacataacagctatacctgtgaggccactcacaagacatcaacttcacccattgtcaagagcttcaacaggaatgagtgtggaggtggatcacttccagaaactggtggaggaagttagagacaaaggtcctgagacgccaccaccagctccccagctccatcctatcttcccttctaaggtcttggaggcttccccacaagcgacctaccactgttgcggtgctccaaacctcctccccacctccttctcctcctcctccctttc

SEQ ID NO: 3 - RNA, 4104 nt, Artificial sequence
  Synthesized
auggauaaaaaauauuccauaggccucgauaucgggacaaauagcgugggcugggcagucaucaccgacgauuauaaggugccuuccaaaaaguuuaagguccuuggaaacacugaccggcacucuaucaaaaaaaaccuuaucggggcccuccuuuuugauucuggugaaaccgcagaagcaaccagauugaaacggacugccagaagacgguacacaaggagaaagaaucggaucugcuaucuucaggaaaucuucagcaacgaaauggccaaaguggacgacucuuucuuucaccgccuggaagagaguuuucuuguggaagaggacaagaaacacgagcgccauccaaucuucgguaacaucguggacgaagucgcuuaucacgagaaauauccaacaaucuaccaccugaggaagaaguuggcugauagcacagacaaggcugaucugagacugaucuaccucgcucucgcucacaugaucaaauuuagaggacacuuccucaucgagggggaccugaacccugacaauagcgacgucgacaagcuguuuauucagcucgugcaaacauacaaucagcuguucgaagagaaccccauuaacgcuucaaggguggaugccaaggcuauucucuccgcacgauugucuaaaagcagacgacuugaaaauuugauugcccagcuuccaggagagaaaaagaacggacuguucgguaaccucauugcucugcuccucggccucaccccaaacuucaagucuaacuucgaccuggcagaggacgcaaagcugcagcucuccaaggacacuuaugaugacgaucuugacaaucugcuggcccagauaggagaccaauaugcugaccuuuuccuugcagccaagaaucugucagaugcaauacugcucagcgacauacuccgggugaacagugaaaucaccaaggcuccauuguccgcauccaugauaaaacgcuacgaugagcaccaccaggacuugacccugcugaaagccuuggugaggcagcagcugcccgaaaaauacaaggagauuuuuuucgaccagaguaagaacggcuaugcaggguauaucgauggaggggcaagucaagaagaauuuuacaaguucaucaaaccuauccuggagaagauggauggaacagaggagcugcuggccaagcuuaacagggaagaccuccugcgcaaacagaggacuuuugauaauggcucuaucccucaucagauccaccugggagagcugcacgcaauccugaggaggcaggaggauuucuauccauuccucaaggauaaucgagagaagaucgagaagauucugacuuuucgcauccccuauuaugucgggccucuggcuagggguaacaguagauuugccuggaugacaaggaagucagaggagaccauuacccccuggaacuuugaagaggugguugacaaaggcgcuagugcccagucuuucauugagagaaugacuaacuucgacaagaaccuuccuaaugagaaagugcucccaaagcauagucugcuguacgaauauuucacuguguacaacgagcuuacaaaggugaaguacgugacagaggguaugaggaaaccugcuuuccuguccggggagcaaaaaaaggccaucguggauuugcuuuucaagacuaaucggaagguuacagucaaacagcugaaagaggauuacuuuaaaaagauugaaugcuuugauucugucgagauuucugguguggaggaccgguucaaugcuagccugggcaccuaccacgaucugcugaagauuaucaaggacaaggacuuccuggacaacgaagagaaugaggacauauuggaggauaucguucucacacucacacuguucgaggacaaggagaugauugaggagaggcugaagaaguaugcacaccuguucgaugauaaagugaugaagcaguugaagagacgacgcuauacuggguggggaaggcugucccgcaagcugauaaacgguauucgagauaagcaauccgguaagaccauccuggauuucuugaaauccgauggauucgcuaaucgaaauuucaugcagcugauucacgacgauagccugacuuucaaggaggacauccagaaggcccagguaagcggccagggugauuccuugcaugaacacauagcaaaucuggccgguuccccugcaaucaagaaggggauccuucagacaguaaaagucguagaugagcuggugaagguaaugggccgacacaagcccgaaaauauugucauugagauggccagggagaaccagacaacucagaagggccagaagaauucccgcgagcgaaugaagcgcauugaggagggaaucaaggaacuugggucugacauucugaaagaauauccaguggagaauacccaacugcagaaugaaaagcuguaccuguauuaucuccaaaacggacgcgacauguauguggaccaagaacuggauaucaacagacuuucagacuacgacguagaucacaucgucccucagagcuuucugaaggacgacucaauugacaacaaggugcuuacccgcagcgacaagaaccgcggcaagucugacaacgucccguccgaggaaguugugaagaaaaugaaaaauuauuggaagcagcugcugaaugcaaaauugaucacucaacggaaauucgauaaucucacaaaagccgaacgaggcggguugucagaacuggacaaagccgguuucaucaagcggcagcuuguggagaccaggcagaucaccaagcacguggcucagauccuggacucccggaugaacacuaaguacgacgagaaugauaagcugauucgagaagugcgcguuaucacacugaaauccaaacugguguccgacuuucgaaaggauuuucaguucuacaagguaagagagauuaacaauuaucaccacgcccaugacgccuaucugaaugcuguggucgguaccgcucucaucaaaaaguacccgaagcuggagucugaguuuguauacggugacuacaaggucuaugaugucaggaagaugaucgccaaaagcgagcaagagauugggaaggcaacagcaaaguacuuuuucuacagcaacaucaugaacuucuuuaaaaccgagauuacacuggccaacggcgagauucgcaaacgcccacugaucgaaacuaauggugagacaggggaaauugugugggauaagggcagagacuucgcuacgguaagaaagguucugucaaugccucaagugaauaucgugaagaaaaccgaagugcagaccggugguuucucuaaggagagcauccuuccgaagcgaaacucugacaaacucaucgcucggaagaaggacugggacccaaagaaguacggaggauuugauagccccacaguggccuacucagugcuggugguggcuaaagucgagaaaggcaaaucuaagaagcugaaauccgugaaagagcugcugggaaucacuauuauggagcgguccaguuucgagaagaacccaaucgacuuccucgaggcuaaagguuacaaagaggugaggaaagauuugauuaucaagcugccaaaguauagccuguucgaacuugagaauggucggaagaggaugcuggcuagcgcuggcgagcuucagaaggggaaugaguuggcuuugcccucaaaguauguuaauuuccucuaucuggcaucacacuacgagaagcugaaggggucccccgaagauaacgaacagaagcagcuuuucguggaacagcacaagcauuaccuggaugagauaaucgaacaaaucucugaguuuagcaagcgcgugauuuuggcugacgcuaaucuugauaaggugcucagugcuuauaacaaacaccgagacaaaccuauaagggaacaagcagagaacaucauccaccucuuuacucugacuaaccugggagccccugccgcauuuaaguauuucgacacaacaauagauaggaagagguauacauccaccaaggaagugcucgacgccacucuuauccaucagaguauuacuggccucuaugaaaccagaaucgaucugagccagcugggcggggac

SEQ ID NO: 4 - RNA, 96 nt, Artificial sequence
  Synthesized
ggaaugaguguuagagacaaguuuuagagcuagaaauagcaaguuaaaauaaggcuaguccguuaucaacuugaaaaaguggcaccgagucggugc

SEQ ID NO: 5 - DNA, 471 bp, Artificial sequence
  Synthesized
atgcaggcaaaaccgcagattccgaaagataaaagcaaagtggccggttatattgaaattccggatgcagatattaaggaaccggtgtatccgggcccggcaacccgcgaacagctgaatcgtggcgtgagttttgccaaagaaaatcagagtctggatgatcagaatattagcattgcaggtcatacctttattgatcgtccgaattatcagtttaccaatctgaaagcagccaaaaaaggtagcatggtttattttaaagtgggcaatgaaacccgtaaatataaaatgaccagtattcgtaacgtgaaaccgaccgcagttgaagtgctggatgaacagaaaggcaaagataaacagctgaccctgattacctgtgatgattataatgaagaaaccggtgtgtgggaaacccgtaagatttttgtggccaccgaagtgaaactcgagcaccaccaccaccaccactga